European Patent Application EP 4 563 590 A1, published June 4, 2025. Title: Composition of Antibacterial Protein for Treating Bovine Mastitis. Applicant: iNtRON Biotechnology, Inc. The sequence listing filed with the application follows.

SEQUENCE LISTING (2 sequences)

SEQ ID NO: 1 - protein, 291 aa, Artificial Sequence
MATYQEYKSRSNGNAYDIDGSFGAQCWDGYADYCKYLGLPYANCTNTGYARDIWEQRHENGILNYFDEVEVMQAGDVAIFMVVDGVTPYSHVAIFDSDAGGGYGWFLGQNQGGANGAYNIVKIPYSATYPTAFRPKVFKNAVTVTGNIGLNKGDYFIDVSAPLPNTAVAPSDSRKPSSKAYYLANDVQLVNDIYQIKCDYLCPVGFDWTENGIPVSLVNWVDENGNHVPDGEDKDFKAGMYFSFEVDEVHITDTGDGGYYGGYYYRSFEFGQFGTVWLSVWDKDDLVNYYN

SEQ ID NO: 2 - DNA, 6106 bp, Artificial Sequence
  source 1..6106: mol_type = other DNA
tggcgaatgggacgcgccctgtagcggcgcattaagcgcggcgggtgtggtggttacgcgcagcgtgaccgctacacttgccagcgccctagcgcccgctcctttcgctttcttcccttcctttctcgccacgttcgccggctttccccgtcaagctctaaatcgggggctccctttagggttccgatttagtgctttacggcacctcgaccccaaaaaacttgattagggtgatggttcacgtagtgggccatcgccctgatagacggtttttcgccctttgacgttggagtccacgttctttaatagtggactcttgttccaaactggaacaacactcaaccctatctcggtctattcttttgatttataagggattttgccgatttcggcctattggttaaaaaatgagctgatttaacaaaaatttaacgcgaattttaacaaaatattaacgtttacaatttcaggtggcacttttcggggaaatgtgcgcggaacccctatttgtttatttttctaaatacattcaaatatgtatccgctcatgaattaattcttagaaaaactcatcgagcatcaaatgaaactgcaatttattcatatcaggattatcaataccatatttttgaaaaagccgtttctgtaatgaaggagaaaactcaccgaggcagttccataggatggcaagatcctggtatcggtctgcgattccgactcgtccaacatcaatacaacctattaatttcccctcgtcaaaaataaggttatcaagtgagaaatcaccatgagtgacgactgaatccggtgagaatggcaaaagtttatgcatttctttccagacttgttcaacaggccagccattacgctcgtcatcaaaatcactcgcatcaaccaaaccgttattcattcgtgattgcgcctgagcgagacgaaatacgcgatcgctgttaaaaggacaattacaaacaggaatcgaatgcaaccggcgcaggaacactgccagcgcatcaacaatattttcacctgaatcaggatattcttctaatacctggaatgctgttttcccggggatcgcagtggtgagtaaccatgcatcatcaggagtacggataaaatgcttgatggtcggaagaggcataaattccgtcagccagtttagtctgaccatctcatctgtaacatcattggcaacgctacctttgccatgtttcagaaacaactctggcgcatcgggcttcccatacaatcgatagattgtcgcacctgattgcccgacattatcgcgagcccatttatacccatataaatcagcatccatgttggaatttaatcgcggcctagagcaagacgtttcccgttgaatatggctcataacaccccttgtattactgtttatgtaagcagacagttttattgttcatgaccaaaatcccttaacgtgagttttcgttccactgagcgtcagaccccgtagaaaagatcaaaggatcttcttgagatcctttttttctgcgcgtaatctgctgcttgcaaacaaaaaaaccaccgctaccagcggtggtttgtttgccggatcaagagctaccaactctttttccgaaggtaactggcttcagcagagcgcagataccaaatactgtccttctagtgtagccgtagttaggccaccacttcaagaactctgtagcaccgcctacatacctcgctctgctaatcctgttaccagtggctgctgccagtggcgataagtcgtgtcttaccgggttggactcaagacgatagttaccggataaggcgcagcggtcgggctgaacggggggttcgtgcacacagcccagcttggagcgaacgacctacaccgaactgagatacctacagcgtgagctatgagaaagcgccacgcttcccgaagggagaaaggcggacaggtatccggtaagcggcagggtcggaacaggagagcgcacgagggagcttccagggggaaacgcctggtatctttatagtcctgtcgggtttcgccacctctgacttgagcgtcgatttttgtgatgctcgtcaggggggcggagcctatggaaaaacgccagcaacgcggcctttttacggttcctggccttttgctggccttttgctcacatgttctttcctgcgttatcccctgattctgtggataaccgtattaccgcctttgagtgagctgataccgctcgccgcagccgaacgaccgagcgcagcgagtcagtgagcgaggaagcggaagagcgcctgatgcggtattttctccttacgcatctgtgcggtatttcacaccgcatatatggtgcactctcagtacaatctgctctgatgccgcatagttaagccagtatacactccgctatcgctacgtgactgggtcatggctgcgccccgacacccgccaacacccgctgacgcgccctgacgggcttgtctgctcccggcatccgcttacagacaagctgtgaccgtctccgggagctgcatgtgtcagaggttttcaccgtcatcaccgaaacgcgcgaggcagctgcggtaaagctcatcagcgtggtcgtgaagcgattcacagatgtctgcctgttcatccgcgtccagctcgttgagtttctccagaagcgttaatgtctggcttctgataaagcgggccatgttaagggcggttttttcctgtttggtcactgatgcctccgtgtaagggggatttctgttcatgggggtaatgataccgatgaaacgagagaggatgctcacgatacgggttactgatgatgaacatgcccggttactggaacgttgtgagggtaaacaactggcggtatggatgcggcgggaccagagaaaaatcactcagggtcaatgccagcgcttcgttaatacagatgtaggtgttccacagggtagccagcagcatcctgcgatgcagatccggaacataatggtgcagggcgctgacttccgcgtttccagactttacgaaacacggaaaccgaagaccattcatgttgttgctcaggtcgcagacgttttgcagcagcagtcgcttcacgttcgctcgcgtatcggtgattcattctgctaaccagtaaggcaaccccgccagcctagccgggtcctcaacgacaggagcacgatcatgcgcacccgtggggccgccatgccggcgataatggcctgcttctcgccgaaacgtttggtggcgggaccagtgacgaaggcttgagcgagggcgtgcaagattccgaataccgcaagcgacaggccgatcatcgtcgcgctccagcgaaagcggtcctcgccgaaaatgacccagagcgctgccggcacctgtcctacgagttgcatgataaagaagacagtcataagtgcggcgacgatagtcatgccccgcgcccaccggaaggagctgactgggttgaaggctctcaagggcatcggtcgagatcccggtgcctaatgagtgagctaacttacattaattgcgttgcgctcactgcccgctttccagtcgggaaacctgtcgtgccagctgcattaatgaatcggccaacgcgcggggagaggcggtttgcgtattgggcgccagggtggtttttcttttcaccagtgagacgggcaacagctgattgcccttcaccgcctggccctgagagagttgcagcaagcggtccacgctggtttgccccagcaggcgaaaatcctgtttgatggtggttaacggcgggatataacatgagctgtcttcggtatcgtcgtatcccactaccgagatatccgcaccaacgcgcagcccggactcggtaatggcgcgcattgcgcccagcgccatctgatcgttggcaaccagcatcgcagtgggaacgatgccctcattcagcatttgcatggtttgttgaaaaccggacatggcactccagtcgccttcccgttccgctatcggctgaatttgattgcgagtgagatatttatgccagccagccagacgcagacgcgccgagacagaacttaatgggcccgctaacagcgcgatttgctggtgacccaatgcgaccagatgctccacgcccagtcgcgtaccgtcttcatgggagaaaataatactgttgatgggtgtctggtcagagacatcaagaaataacgccggaacattagtgcaggcagcttccacagcaatggcatcctggtcatccagcggatagttaatgatcagcccactgacgcgttgcgcgagaagattgtgcaccgccgctttacaggcttcgacgccgcttcgttctaccatcgacaccaccacgctggcacccagttgatcggcgcgagatttaatcgccgcgacaatttgcgacggcgcgtgcagggccagactggaggtggcaacgccaatcagcaacgactgtttgcccgccagttgttgtgccacgcggttgggaatgtaattcagctccgccatcgccgcttccactttttcccgcgttttcgcagaaacgtggctggcctggttcaccacgcgggaaacggtctgataagagacaccggcatactctgcgacatcgtataacgttactggtttcacattcaccaccctgaattgactctcttccgggcgctatcatgccataccgcgaaaggttttgcgccattcgatggtgtccgggatctcgacgctctcccttatgcgactcctgcattaggaagcagcccagtagtaggttgaggccgttgagcaccgccgccgcaaggaatggtgcatgcaaggagatggcgcccaacagtcccccggccacggggcctgccaccatacccacgccgaaacaagcgctcatgagcccgaagtggcgagcccgatcttccccatcggtgatgtcggcgatataggcgccagcaaccgcacctgtggcgccggtgatgccggccacgatgcgtccggcgtagaggatcgagatctcgatcccgcgaaattaatacgactcactataggggaattgtgagcggataacaattcccctctagaaataattttgtttaactttaagaaggagatataccatggctacgtatcaggagtataaatcgcggagcaatggcaacgcctatgatattgacggttcttttggtgcacagtgttgggacgggtatgcagactactgtaaatatttggggctgccttacgccaactgtacaaacaccggttacgcccgtgatatctgggaacagcgtcacgagaatggcatcctgaactattttgacgaggtagaagtgatgcaagctggggatgttgcaatctttatggtggtggacggggttacaccatattcacacgtcgctatcttcgatagtgacgcaggtggcggctacggttggtttttaggccagaatcaagggggtgccaatggcgcctacaacatcgtcaaaattccttatagtgcaacatatcctactgcattccgtccaaaggttttcaaaaacgctgtcaccgttacaggcaatattgggttgaacaagggggactacttcattgacgtctcagccccattgccgaataccgcagtagcaccatcagattcccgcaaacctagcagtaaagcgtactaccttgcaaacgacgttcaattagtgaatgacatttaccagatcaagtgcgactatctgtgtccggttgggttcgattggaccgagaatggtattccagtatccttagtaaattgggtcgatgaaaacggcaatcacgtacctgatggtgaggataaagattttaaggccgggatgtatttctctttcgaggtagatgaggtacacattacagatacgggtgatggcggctattatggcggctattactatcgtagcttcgaattcgggcagtttgggacagtgtggttaagcgtttgggacaaagatgatctcgtaaactactataatctcgagcaccaccaccaccaccactgagatccggctgctaacaaagcccgaaaggaagctgagttggctgctgccaccgctgagcaataactagcataaccccttggggcctctaaacgggtcttgaggggttttttgctgaaaggaggaactatatccggat